European Patent Specification EP 3 360 896 B1, published July 23, 2025. Title: Antibody against hepatitis B surface antigen and use thereof. Applicant: XIAMEN UNIVERSITY; YANG SHENG TANG COMPANY,LTD. Application 2016-10-09. The sequence listing filed with the application follows.

SEQUENCE LISTING (320 sequences)

SEQ ID NO: 1 - protein, 113 aa, Artificial Sequence
DVQLQESGPGLVKPSQSLSLTCSVTGYPITSGYHWNWIRQFPGNKLVWMGYISYDGSDHYNPSLENRISITRDISKNQFFLILRSVTTEDTGKYFCASGFDHWGQGTTLTVSS

SEQ ID NO: 2 - protein, 113 aa, Artificial Sequence
DVVMTQTPLSLPVSLGDQASISCRSSQSLVHSYGDTYLHWYLQKPGQSPKLLIYKVSNRFSGVPDRFSGSGSGTDFTLKISRVETEDLGVYFCSQNTHVPYTFGGGTKLEIKR

SEQ ID NO: 3 - protein, 6 aa, Artificial Sequence
SGYHWN

SEQ ID NO: 4 - protein, 16 aa, Artificial Sequence
YISYDGSDHYNPSLEN

SEQ ID NO: 5 - protein, 4 aa, Artificial Sequence
GFDH

SEQ ID NO: 6 - protein, 16 aa, Artificial Sequence
RSSQSLVHSYGDTYLH

SEQ ID NO: 7 - protein, 7 aa, Artificial Sequence
KVSNRFS

SEQ ID NO: 8 - protein, 9 aa, Artificial Sequence
SQNTHVPYT

SEQ ID NO: 9 - protein, 98 aa, Artificial Sequence
QVQLQESGPGLVKPSQTLSLTCAVSGYSISSSNWWGWIRQPPGKGLEWIGYIYYSGSIYYNPSLKSRVTMSVDTSKNQFSLKLSSVTAVDTAVYYCAR

SEQ ID NO: 10 - protein, 93 aa, Artificial Sequence
DIVMTQSPLSLPVTPGEPASISCRSSQSLLHSNGYNYLDWYLQKPGQSPQLLIYLGSNRASGVPDRFSGSGSGTDFTLKISRVEAEDVGVYYC

SEQ ID NO: 11 - protein, 113 aa, Artificial Sequence
EVQLQESGPGLVKPSQTLSLTCAVSGYSISSGYHWNWIRQFPGNKLEWIGYISYDGSDHYNPSLENRITITRDTSKNQFSLILRSVTAEDTAIYYCASGFDHWGQGTTLTVSS

SEQ ID NO: 12 - protein, 113 aa, Artificial Sequence
EVQLQESGPGLVKPSQTLSLTCAVSGYSISRGYHWNWIRQFPGNKLEWIGYISYDGSVFYNPSLENRVTITRDTSKNQFFLKLSSVTAEDTAKYYCASGFDYWGQGTTLTVSS

SEQ ID NO: 13 - protein, 113 aa, Artificial Sequence
EVQLQESGPGLVKPSQTLSLTCAVSGYSISHGYHWNWIRQFPGNKLEWIGYISYDGSILYNPSLENRVTITRDTSKNQFFLKLSSVTAEDTAKYYCASGFDHWGQGTTLTVSS

SEQ ID NO: 14 - protein, 113 aa, Artificial Sequence
EVQLQESGPGLVKPSQTLSLTCAVSGYSITNGYHWNWIRQFPGNKLEWIGYISYDGTILYNPSLENRVTITRDTSKNQFFLKLSSVTAEDTAKYYCASGFDHWGQGTTLTVSS

SEQ ID NO: 15 - protein, 113 aa, Artificial Sequence
EVQLQESGPGLVKPSQTLSLTCAVSGTSITRGYHWNWIRQFPGNKLEWIGYISYDGSILYNPSLENRVTITRDTSKNQFFLKLSSVTAEDTAKYYCASGFDHWGQGTTLTVSS

SEQ ID NO: 16 - protein, 113 aa, Artificial Sequence
EVQLQESGPGLVKPSQTLSLTCAVSGTSITHGYHWNWIRQFPGNKLEWIGYISYDGTVLYNPSLENRVTITRDTSKNQFFLKLSSVTAEDTAKYYCASGFDYWGQGTTLTVSS

SEQ ID NO: 17 - protein, 113 aa, Artificial Sequence
EVQLQESGPGLVKPSQTLSLTCAVSGYSISSGYHWNWIRQFPGNKLEWIGYISYDGSILYNPSLENRVTITRDTSKNQFFLKLSSVTAEDTAKYYCASGFDHWGQGTTLTVSS

SEQ ID NO: 18 - protein, 113 aa, Artificial Sequence
EVQLQESGPGLVKPSQTLSLTCAVSGTSITRDYHWNWIRQFPGNKLEWIGYISYDGTVLYNPSLENRVTITRDTSKNQFFLKLSSVTAEDTAKYYCASGFDYWGQGTTLTVSS

SEQ ID NO: 19 - protein, 113 aa, Artificial Sequence
EVQLQESGPGLVKPSQTLSLTCAVSGYSISSGYHWNWIRQFPGNKLEWIGYISYDGNVLYNPSLENRVTITRDTSKNQFFLKLSSVTAEDTAKYYCASGFDYWGQGTTLTVSS

SEQ ID NO: 20 - protein, 113 aa, Artificial Sequence
EVQLQESGPGLVKPSQTLSLTCAVSGNSISRWYHWNWIRQFPGNKLEWIGYISYDGTVLYNPSLENRVTITRDTSKNQFFLKLSSVTAEDTAKYYCASGFDHWGQGTTLTVSS

SEQ ID NO: 21 - protein, 113 aa, Artificial Sequence
EVQLQESGPGLVKPSQTLSLTCAVSGYSISHGYHWNWIRQFPGNKLEWIGYISYDGTVLYNPSLENRVTITRDTSKNQFFLKLSSVTAEDTAKYYCASGFDHWGQGTTLTVSS

SEQ ID NO: 22 - protein, 113 aa, Artificial Sequence
EVQLQESGPGLVKPSQTLSLTCAVSGASITRDYHWNWIRQFPGNKLEWIGYISYDGTILYNPSLENRVTITRDTSKNQFFLKLSSVTAEDTAKYYCASGFDHWGQGTTLTVSS

SEQ ID NO: 23 - protein, 113 aa, Artificial Sequence
EVQLQESGPGLVKPSQTLSLTCAVSGYSISHGYHWNWIRQFPGNKLEWIGYISYDGTILYNPSLENRVTITRDTSKNQFFLKLSSVTAEDTAKYYCASGFDHWGQGTTLTVSS

SEQ ID NO: 24 - protein, 113 aa, Artificial Sequence
EVQLQESGPGLVKPSQTLSLTCAVSGASITYGYHWNWIRQFPGNKLEWIGYISYDGSILYNPSLENRVTITRDTSKNQFFLKLSSVTAEDTAKYYCASGFDYWGQGTTLTVSS

SEQ ID NO: 25 - protein, 113 aa, Artificial Sequence
EVQLQESGPGLVKPSQTLSLTCAVSGASITHGYHWNWIRQFPGNKLEWIGYISYDGTSLYNPSLENRVTITRDTSKNQFFLKLSSVTAEDTAKYYCASGFDHWGQGTTLTVSS

SEQ ID NO: 26 - protein, 113 aa, Artificial Sequence
EVQLQESGPGLVKPSQTLSLTCAVSGASITRGYHWNWIRQFPGNKLEWIGYISYDGTVLYNPSLENRVTITRDTSKNQFFLKLSSVTAEDTAKYYCASGFDYWGQGTTLTVSS

SEQ ID NO: 27 - protein, 113 aa, Artificial Sequence
EVQLQESGPGLVKPSQTLSLTCAVSGYSISSGYHWNWIRQFPGNKLEWIGYISYDGTILYNPSLENRVTITRDTSKNQFFLKLSSVTAEDTAKYYCASGFDYWGQGTTLTVSS

SEQ ID NO: 28 - protein, 113 aa, Artificial Sequence
EVQLQESGPGLVKPSQTLSLTCAVSGTSITRGYHWNWIRQFPGNKLEWIGYISYDGSILYNPSLENRVTITRDTSKNQFFLKLSSVTAEDTAKYYCASGFDYWGQGTTLTVSS

SEQ ID NO: 29 - protein, 113 aa, Artificial Sequence
EVQLQESGPGLVKPSQTLSLTCAVSGASITYGYHWNWIRQFPGNKLEWIGYISYDGTILYNPSLENRVTITRDTSKNQFFLKLSSVTAEDTAKYYCASGFDTWGQGTTLTVSS

SEQ ID NO: 30 - protein, 113 aa, Artificial Sequence
EVQLQESGPGLVKPSQTLSLTCAVSGSSITNFYHWNWIRQFPGNKLEWIGYISYDGSVLYNPSLENRVTITRDTSKNQFFLKLSSVTAEDTAKYYCASGFDHWGQGTTLTVSS

SEQ ID NO: 31 - protein, 113 aa, Artificial Sequence
EVQLQESGPGLVKPSQTLSLTCAVSGASITYGYHWNWIRQFPGNKLEWIGYISYDGTILYNPSLENRVTITRDTSKNQFFLKLSSVTAEDTAKYYCASGFDHWGQGTTLTVSS

SEQ ID NO: 32 - protein, 113 aa, Artificial Sequence
EVQLQESGPGLVKPSQTLSLTCAVSGSSITRGYHWNWIRQFPGNKLEWIGYISYDGTILYNPSLENRVTITRDTSKNQFFLKLSSVTAEDTAKYYCASGFDHWGQGTTLTVSS

SEQ ID NO: 33 - protein, 113 aa, Artificial Sequence
EVQLQESGPGLVKPSQTLSLTCAVSGASITHGYHWNWIRQFPGNKLEWIGYISYDGTILYNPSLENRVTITRDTSKNQFFLKLSSVTAEDTAKYYCASGFDYWGQGTTLTVSS

SEQ ID NO: 34 - protein, 113 aa, Artificial Sequence
EVQLQESGPGLVKPSQTLSLTCAVSGTSITSGYHWNWIRQFPGNKLEWIGYISYDGTVLYNPSLENRVTITRDTSKNQFFLKLSSVTAEDTAKYYCASGFDHWGQGTTLTVSS

SEQ ID NO: 35 - protein, 113 aa, Artificial Sequence
EVQLQESGPGLVKPSQTLSLTCAVSGYSISSGYHWNWIRQFPGNKLEWIGYISYDGTILYNPSLENRVTITRDTSKNQFFLKLSSVTAEDTARYYCASGFDHWGQGTTLTVSS

SEQ ID NO: 36 - protein, 113 aa, Artificial Sequence
EVQLQESGPGLVKPSQTLSLTCAVSGSSITYGYHWNWIRQFPGNKLEWIGYISYDGSVLYNPSLENRVTITRDTSKNQFFLKLSSVTAEDTAKYYCASGFDHWGQGTTLTVSS

SEQ ID NO: 37 - protein, 113 aa, Artificial Sequence
EVQLQESGPGLVKPSQTLSLTCAVSGTSITRGYHWNWIRQFPGNKLEWIGYISYDGNILYNPSLENRVTITRDTSKNQFFLKLSSVTAEDTAKYYCASGFDYWGQGTTLTVSS

SEQ ID NO: 38 - protein, 113 aa, Artificial Sequence
EVQLQESGPGLVKPSQTLSLTCAVSGYSISSGYHWNWVRQFPGNKLEWIGYISYDGTNLYNPSLENRVTITRDTSKNQFFLKLSSVTAEDTAKYYCASGFDHWGQGTTLTVSS

SEQ ID NO: 39 - protein, 113 aa, Artificial Sequence
EVQLQESGPGLVKPSQTLSLTCAVSGASITHGYHWNWIRQFPGNKLEWIGYISYDGTVLYNPSLENRVTITRDTSKNQFFLKLSSVTAEDTAKYYCASGFDHWGQGTTLTVSS

SEQ ID NO: 40 - protein, 113 aa, Artificial Sequence
EVQLQESGPGLVKPSQTLSLTCAVSGASITHGYHWNWIRQFPGNKLEWIGYISYDGSNLYNPSLENRVTITRDTSKNQFFLKLSSVTAEDTAKYYCASGFDYWGQGTTLTVSS

SEQ ID NO: 41 - protein, 113 aa, Artificial Sequence
EVQLQESGPGLVKPSQTLSLTCAVSGYSITRGYHWNWIRQFPGNKLEWIGYISYDGTNLYNPSLENRVTITRDTSKNQFFLKLSSVTAEDTAKYYCASGFDHWGQGTTLTVSS

SEQ ID NO: 42 - protein, 113 aa, Artificial Sequence
EVQLQESGPGLVKPSQTLSLTCAVSGSSITHGYHWNWIRQFPGNKLEWIGYISYDGTILYNPSLENRVTITRDTSKNQFFLKLSSVTAEDTAKYYCASGFDHWGQGTTLTVSS

SEQ ID NO: 43 - protein, 113 aa, Artificial Sequence
EVQLQESGPGLVKPSQTLSLTCAVSGYSISSGYHWNWIRQFPGNKLEWIGYISYDGSILYNPSLENRVTITRDTSKNQFFLKLSSVTAEDTAKYYCASGFDYWGQGTTLTVSS

SEQ ID NO: 44 - protein, 113 aa, Artificial Sequence
EVQLQESGPGLVKPSQTLSLTCAVSGASISYGYHWNWIRQFPGNKLEWIGYISYDGTVHYNPSLENRVTITRDTSKNQFFLKLSSVTAEDTAKYYCASGFDHWGQGTTLTVSS

SEQ ID NO: 45 - protein, 113 aa, Artificial Sequence
EVQLQESGPGLVKPSQTLSLTCAVSGTSITNFYHWNWIRQFPGNKLEWIGYISYDGNVLYNPSLENRVTITRDTSKNQFFLKLSSVTAEDTAKYYCASGFDYWGQGTTLTVSS

SEQ ID NO: 46 - protein, 113 aa, Artificial Sequence
EVQLQESGPGLVKPSQTLSLTCAVSGASITRDYHWNWIQQFPGNKLEWIGYISYDGTILYNPSLENRVTITRDTSKNQFFLKLSSVTAEDTAKYYCASGFDHWGQGTTLTVSS

SEQ ID NO: 47 - protein, 113 aa, Artificial Sequence
EVQLQESGPGLVKPSQTLSLTCAVSGTSITRYYHWNWIRQFPGNKLEWIGYISYDGTIRYNPSLENRVTITRDTSKNQFFLKLSSVTAEDTAKYYCASGFDHWGQGTTLTVSS

SEQ ID NO: 48 - protein, 113 aa, Artificial Sequence
EVQLQESGPGLVKPSQTLSLTCAVSGSSITYGYHWNWIRQFPGNKLEWIGYISYDGTVHYNPSLENRVTITRDTSKNQFFLKLSSVTAEDTAKYYCASGFDYWGQGTTLTVSS

SEQ ID NO: 49 - protein, 113 aa, Artificial Sequence
EVQLQESGPGLVKPSQTLSLTCAVSGGSITRDYHWNWIRQFPGNKLEWIGYISYDGTVLYNPSLENRVTITRDTSKNQFFLKLSSVTAEDTAKYYCASGFDHWGQGTTLTVSS

SEQ ID NO: 50 - protein, 113 aa, Artificial Sequence
EVQLQESGPGLVKASQTLSLTCAVSGYSISSGYHWNWIRQLPGNKLEWIGYISYDGSDHYNPSLENRITISRDTSKNQFFLKLRSVTAEDTAKYFCASGFDHWGQGTTLTVSS

SEQ ID NO: 51 - protein, 113 aa, Artificial Sequence
DVQLQESGPGLVKPSQTLSLTCAVSGYPITSGYHWNWIRQFPGNKLEWIGYISYDGSDHYNPSLENRVSITRDTSKNQFFLILRSVTAEDTAIYYCASGFDHWGQGTTLTVSS

SEQ ID NO: 52 - protein, 113 aa, Artificial Sequence
HVQLQESGPGLVKPSQTLSLTCAVSGYSITSGYHWNWIRQFPGNKLEWIGYISYDGSDHYNPSLENRVTITRDTSKNQFFLKLRSVTAEDTAIYYCASGFDHWGQGTTLTVSS

SEQ ID NO: 53 - protein, 113 aa, Artificial Sequence
EVQLQESGPGLVKPSQTLSLTCAVSGYSITSGYHWNWIRQFPGNKLEWIGYISYDGSDHYNPSLENRVSITRDTSKNQFFLKLSSVTAEDTAKYFCASGFDHWGQGTTLTVSS

SEQ ID NO: 54 - protein, 113 aa, Artificial Sequence
EVQLQESGPGLVKPSQTLSLTCAVSGYPISSGYHWNWIRQFPGKKLEWIGYISYDGSDHYNPSLENRVTITRDTSKNQFFLKLRSVTAEDTAIYFCASGFDHWGQGTTLTVSS

SEQ ID NO: 55 - protein, 113 aa, Artificial Sequence
QVQLQESGPGLVKPSQTLSLTCAVSGYSISYGYHWNWIRQFPGKGLEWIGYISYDGSVLYNPSLKSRVTISVDTSKNQFSLKLSSVTAEDTAVYYCASGFDHWGQGTLVTVSS

SEQ ID NO: 56 - protein, 113 aa, Artificial Sequence
HVQLQESGPGLVKPSQTLSLTCAVSGTSITRGYHWNWIRQFPGNKLEWIGYISYDGSILYNPSLENRVTITRDTSKNQFFLKLRSVTAEDTAIYYCASGFDHWGQGTTLTVSS

SEQ ID NO: 57 - protein, 113 aa, Artificial Sequence
HVQLQESGPGLVKPSQTLSLTCAVSGNSISRWYHWNWIRQFPGNKLEWIGYISYDGTVLYNPSLENRVTITRDTSKNQFFLKLRSVTAEDTAIYYCASGFDHWGQGTTLTVSS

SEQ ID NO: 58 - protein, 113 aa, Artificial Sequence
HVQLQESGPGLVKPSQTLSLTCAVSGYSISHGYHWNWIRQFPGNKLEWIGYISYDGTVLYNPSLENRVTITRDTSKNQFFLKLRSVTAEDTAIYYCASGFDHWGQGTTLTVSS

SEQ ID NO: 59 - protein, 113 aa, Artificial Sequence
HVQLQESGPGLVKPSQTLSLTCAVSGASITRDYHWNWIRQFPGNKLEWIGYISYDGTILYNPSLENRVTITRDTSKNQFFLKLRSVTAEDTAIYYCASGFDHWGQGTTLTVSS

SEQ ID NO: 60 - protein, 113 aa, Artificial Sequence
HVQLQESGPGLVKPSQTLSLTCAVSGSSITYGYHWNWIRQFPGNKLEWIGYISYDGSVLYNPSLENRVTITRDTSKNQFFLKLRSVTAEDTAIYYCASGFDHWGQGTTLTVSS

SEQ ID NO: 61 - protein, 113 aa, Artificial Sequence
HVQLQESGPGLVKPSQTLSLTCAVSGASITRWYHWNWIRQFPGNKLEWIGYISYDGTVLYNPSLENRVTITRDTSKNQFFLKLRSVTAEDTAIYYCASGFDYWGQGTTLTVSS

SEQ ID NO: 62 - protein, 113 aa, Artificial Sequence
DVQLQESGPGLVKPSQTLSLTCAVSGYSITNGYHWNWIRQFPGNKLEWIGYISYDGTILYNPSLENRVSITRDTSKNQFFLILRSVTAEDTAIYYCASGFDHWGQGTTLTVSS

SEQ ID NO: 63 - protein, 113 aa, Artificial Sequence
DVQLQESGPGLVKPSQTLSLTCAVSGYSISHGYHWNWIRQFPGNKLEWIGYISYDGTILYNPSLENRVSITRDTSKNQFFLILRSVTAEDTAIYYCASGFDHWGQGTTLTVSS

SEQ ID NO: 64 - protein, 113 aa, Artificial Sequence
DVQLQESGPGLVKPSQTLSLTCAVSGTSITRGYHWNWIRQFPGNKLEWIGYISYDGSILYNPSLENRVSITRDTSKNQFFLILRSVTAEDTAIYYCASGFDHWGQGTTLTVSS

SEQ ID NO: 65 - protein, 113 aa, Artificial Sequence
DVQLQESGPGLVKPSQTLSLTCAVSGNSISRWYHWNWIRQFPGNKLEWIGYISYDGTVLYNPSLENRVSITRDTSKNQFFLILRSVTAEDTAIYYCASGFDHWGQGTTLTVSS

SEQ ID NO: 66 - protein, 113 aa, Artificial Sequence
DVQLQESGPGLVKPSQTLSLTCAVSGSSITYGYHWNWIRQFPGNKLEWIGYISYDGSVLYNPSLENRVSITRDTSKNQFFLILRSVTAEDTAIYYCASGFDHWGQGTTLTVSS

SEQ ID NO: 67 - protein, 113 aa, Artificial Sequence
DVQLQESGPGLVKPSQTLSLTCAVSGYSITRGYHWNWIRQFPGNKLEWIGYISYDGTNLYNPSLENRVSITRDTSKNQFFLILRSVTAEDTAIYYCASGFDHWGQGTTLTVSS

SEQ ID NO: 68 - protein, 113 aa, Artificial Sequence
HVQLQESGPGLVKPSQTLSLTCAVSGYSISHGYHWNWIRQFPGNKLEWIGYISYDGTILYNPSLENRVTITRDTSKNQFFLKLRSVTAEDTAIYYCASGFDHWGQGTTLTVSS

SEQ ID NO: 69 - protein, 113 aa, Artificial Sequence
DVQLQESGPGLVKPSQTLSLTCTVSGYPITSGYHWNWIRQFPGNKLVWMGYISYDGSDHYNPSLENRVSISRDISKNQFFLKLSSVTAADTAVYFCASGFDHWGQGTMLTVSS

SEQ ID NO: 70 - protein, 113 aa, Artificial Sequence
QVQLQESGPGLVKPSQTLSLTCAVSGYSISYGYHWNWIRQFPGKGLEWIGYISYDGSVLYNPSLKGRVTISVDTSKNQFSLKLSSVTAEDTAVYYCASGFDHWGQGTLVTVSS

SEQ ID NO: 71 - protein, 113 aa, Artificial Sequence
QVQLQESGPGLVKPSQTLSLTCAVSGYSISNGYHWNWIRQFPGKSLEWIGYIAYDGVQSYNPSLKGRVTISVDTSKNQFSLKLSSVTAEDTAVYYCASGFDHWGQGTLVTVSS

SEQ ID NO: 72 - protein, 113 aa, Artificial Sequence
QVQLQESGPGLVKPSQTLSLTCAVSGYSISRGYHWNWIRQFPGKGLEWIGYISYDGSVLYNPSLKSRVTISVDTSKNQFSLKLSSVTAEDTAVYYCASGFDHWGQGTLVTVSS

SEQ ID NO: 73 - protein, 113 aa, Artificial Sequence
QVQLQESGPGLVKPSQTLSLTCAVSGYSISSGYHWNWIRQFPGKGLEWIGYISYDGSVLYNPSLKSRVTISVDTSKNQFSLKLSSVTAEDTAVYYCASGFDHWGQGTLVTVSS

SEQ ID NO: 74 - protein, 113 aa, Artificial Sequence
QVQLQESGPGLVKPSQTLSLTCAVSGYSISNGYHWNWIRQFPGKGLEWIGYISYDGSVLYNPSLKSRVTISVDTSKNQFSLKLSSVTAEDTAVYYCASGFDHWGQGTLVTVSS

SEQ ID NO: 75 - protein, 113 aa, Artificial Sequence
QVQLQESGPGLVKPSQTLSLTCAVSGYSISRGYHWNWIRQFPGKGLEWIGYIGYDGAVQYNPSLKSRVTISVDTSKNQFSLKLSSVTAEDTAVYYCASGFDHWGQGTLVTVSS

SEQ ID NO: 76 - protein, 113 aa, Artificial Sequence
QVQLQESGPGLVKPSQTLSLTCAVSGYSISHGYHWNWIRQFPGKSLEWIGYISYNGSVLYNPSLKSRVTISVDTSKNQFSLKLSSVTAEDTAVYYCASGFDHWGQGTLVTVSS

SEQ ID NO: 77 - protein, 113 aa, Artificial Sequence
QVQLQESGPGLVKPSQTLSLTCAVSGYSISRGYHWNWIRQFPGKGLEWIGYISYDGSRLYNPSLKSRVTISVDTSKNQFSLKLSSVTAEDTAVYYCASGFDHWGQGTLVTVSS

SEQ ID NO: 78 - protein, 113 aa, Artificial Sequence
QVQLQESGPGLVKPSQTLSLTCAVSGYSISNGYHWNWIRQFPGKGLEWIGYISYNGSVLYNPSLKSRVTISVDTSKNQFSLKLSSVTAEDTAVYYCASGFDHWGQGTLVTVSS

SEQ ID NO: 79 - protein, 113 aa, Artificial Sequence
EVQLQESGPGLVKPSQTLSLTCAVSGYSITSGYHWNWIRQFPGKRLEWMGYISYDGSDHYNPSLENRITITRDTSKNQFFLKLRSVTAEDTAVYYCASGFDHWGQGTTLTVSS

SEQ ID NO: 80 - protein, 113 aa, Artificial Sequence
EVQLQESGPGLVKPSQTLSLTCAVSGYPITSGYHWNWIRQFPGNKLEWIGYISYDGSDHYNPSLENRVSITRDTSKNQFFLKLRSVTAEDTAIYFCASGFDHWGQGTTLTVSS

SEQ ID NO: 81 - protein, 113 aa, Artificial Sequence
EVQLQESGPGLVKPSQTLSLTCAVSGYSITSGYHWNWIRQFPGNELEWIGYISYDGSDHYNPSLENRITITRDTSKNQFFLKLRSVTAEDTAKYYCASGFDHWGQGTTLTVSS

SEQ ID NO: 82 - protein, 113 aa, Artificial Sequence
HVQLQESGPGLVKPSQTLSLTCAVSGYSITNGYHWNWIRQFPGNKLEWIGYISYDGTILYNPSLENRVTITRDTSKNQFFLKLRSVTAEDTAIYYCASGFDHWGQGTTLTVSS

SEQ ID NO: 83 - protein, 113 aa, Artificial Sequence
EVQLQESGPGLVKPSQTLSLTCAVSGYSISSGYHWNWIRQFPGNRLEWIGYISYDGSDHYNPSLENRVTITRDTSKNQFFLILRSVTAEDTAKYYCASGFDHWGQGTTLTVSS

SEQ ID NO: 84 - protein, 113 aa, Artificial Sequence
EVQLQESGPGLVKPSQTLSLTCAVSGYSITSGYHWNWIRQFPGNKLEWIGYISYDGSDHYNPSLENRVTITRDTSKNQFFLKLRSVTAEDTAKYYCASGFDHWGQGTTLTVSS

SEQ ID NO: 85 - protein, 113 aa, Artificial Sequence
QVQLQESGPGLVKPSQTLSLTCAVSGYSISSGYHWNWIRQFPGNRLEWMGYISYDGSDHYNPSLENRISITRDTSKNQFFLKLSSVTAEDTAKYFCASGFDHWGQGTTLTVSS

SEQ ID NO: 86 - protein, 113 aa, Artificial Sequence
EVQLQESGPGLVKPSQTLSLTCAVSGYSITSGYHWNWIRQFPGNKLEWIGYISYDGSDHYNPSLENRITITRDTSKNQFSLKLRSVTAEDTAVYYCASGFDHWGQGTTLTVSS

SEQ ID NO: 87 - protein, 113 aa, Artificial Sequence
EVQLQESGPGLVKPSQTLSLTCAVSGYSITSGYHWNWIRQFPGNKLEWIGYISYDGSDHYNPSLENRVTITRDTSKNQFFLKLSSVTAEDTAKYYCASGFDHWGQGTTLTVSS

SEQ ID NO: 88 - protein, 113 aa, Artificial Sequence
QVQQQESGPGQVKPSQTLSLTCAVSGYPISSGYHWNWIRQFPGNKLEWMGYISYDGSDHYNPSLENRITITRDTSKNQFFLKLRSVTAEDTAKYYCASGFDHWGQGTTLTVSS

SEQ ID NO: 89 - protein, 113 aa, Artificial Sequence
QVQLQESGPGLVKPSQTLSLTCAVSGYSITSGYHWNWIRQFPGNKLEWMGYISYDGSDHYNPSLENRITITRDTSKNQFFLILRSVTAEDTAIYYCASGFDHWGQGTTLTVSS

SEQ ID NO: 90 - protein, 113 aa, Artificial Sequence
HVQLQESGPGLVKPSQTLSLTCAVSGYSISSGYHWNWIRQFPGNELEWIGYISYDGSDHYNPSLENRITITRDTSKNQFFLKLRSVTAEDTAKYYCASGFDHWGQGTTLTVSS

SEQ ID NO: 91 - protein, 113 aa, Artificial Sequence
QVQLQESGPGLVKPSQTLSLTCAVSGYSISRGYHWNWIRQFPGKGLEWIGYISYDGSVLYNPSLKSRVTISVDTSKNQFSLKLSSVTTEDTAVYYCASGFDHWGQGTLVTVSS

SEQ ID NO: 92 - protein, 113 aa, Artificial Sequence
QVQLQESGPGLVKPSQTLSLTCAVSGYSISHGYHWNWIRQFPGKGLEWIGYISYDGSVLYNPSLKSRVTISVDTSKNQFSLKLSSVTAEDTAVYYCASGFDHWGQGTLVTVSS

SEQ ID NO: 93 - protein, 30 aa, Artificial Sequence
EVQLQESGPGLVKPSQTLSLTCAVSGYSIS

SEQ ID NO: 94 - protein, 30 aa, Artificial Sequence
EVQLQESGPGLVKPSQTLSLTCAVSGYSIT

SEQ ID NO: 95 - protein, 30 aa, Artificial Sequence
EVQLQESGPGLVKPSQTLSLTCAVSGTSIT

SEQ ID NO: 96 - protein, 30 aa, Artificial Sequence
EVQLQESGPGLVKPSQTLSLTCAVSGNSIS

SEQ ID NO: 97 - protein, 30 aa, Artificial Sequence
EVQLQESGPGLVKPSQTLSLTCAVSGASIT

SEQ ID NO: 98 - protein, 30 aa, Artificial Sequence
EVQLQESGPGLVKPSQTLSLTCAVSGSSIT

SEQ ID NO: 99 - protein, 30 aa, Artificial Sequence
EVQLQESGPGLVKPSQTLSLTCAVSGASIS

SEQ ID NO: 100 - protein, 30 aa, Artificial Sequence
EVQLQESGPGLVKPSQTLSLTCAVSGGSIT

SEQ ID NO: 101 - protein, 30 aa, Artificial Sequence
EVQLQESGPGLVKASQTLSLTCAVSGYSIS

SEQ ID NO: 102 - protein, 30 aa, Artificial Sequence
DVQLQESGPGLVKPSQTLSLTCAVSGYPIT

SEQ ID NO: 103 - protein, 30 aa, Artificial Sequence
HVQLQESGPGLVKPSQTLSLTCAVSGYSIT

SEQ ID NO: 104 - protein, 30 aa, Artificial Sequence
EVQLQESGPGLVKPSQTLSLTCAVSGYPIS

SEQ ID NO: 105 - protein, 30 aa, Artificial Sequence
QVQLQESGPGLVKPSQTLSLTCAVSGYSIS

SEQ ID NO: 106 - protein, 30 aa, Artificial Sequence
HVQLQESGPGLVKPSQTLSLTCAVSGTSIT

SEQ ID NO: 107 - protein, 30 aa, Artificial Sequence
HVQLQESGPGLVKPSQTLSLTCAVSGNSIS

SEQ ID NO: 108 - protein, 30 aa, Artificial Sequence
HVQLQESGPGLVKPSQTLSLTCAVSGYSIS

SEQ ID NO: 109 - protein, 30 aa, Artificial Sequence
HVQLQESGPGLVKPSQTLSLTCAVSGASIT

SEQ ID NO: 110 - protein, 30 aa, Artificial Sequence
HVQLQESGPGLVKPSQTLSLTCAVSGSSIT

SEQ ID NO: 111 - protein, 30 aa, Artificial Sequence
DVQLQESGPGLVKPSQTLSLTCAVSGYSIT

SEQ ID NO: 112 - protein, 30 aa, Artificial Sequence
DVQLQESGPGLVKPSQTLSLTCAVSGYSIS

SEQ ID NO: 113 - protein, 30 aa, Artificial Sequence
DVQLQESGPGLVKPSQTLSLTCAVSGTSIT

SEQ ID NO: 114 - protein, 30 aa, Artificial Sequence
DVQLQESGPGLVKPSQTLSLTCAVSGNSIS

SEQ ID NO: 115 - protein, 30 aa, Artificial Sequence
DVQLQESGPGLVKPSQTLSLTCAVSGSSIT

SEQ ID NO: 116 - protein, 30 aa, Artificial Sequence
DVQLQESGPGLVKPSQTLSLTCTVSGYPIT

SEQ ID NO: 117 - protein, 30 aa, Artificial Sequence
EVQLQESGPGLVKPSQTLSLTCAVSGYPIT

SEQ ID NO: 118 - protein, 30 aa, Artificial Sequence
QVQQQESGPGQVKPSQTLSLTCAVSGYPIS

SEQ ID NO: 119 - protein, 30 aa, Artificial Sequence
QVQLQESGPGLVKPSQTLSLTCAVSGYSIT

SEQ ID NO: 120 - protein, 6 aa, Artificial Sequence
SGYHWN

SEQ ID NO: 121 - protein, 6 aa, Artificial Sequence
RGYHWN

SEQ ID NO: 122 - protein, 6 aa, Artificial Sequence
HGYHWN

SEQ ID NO: 123 - protein, 6 aa, Artificial Sequence
NGYHWN

SEQ ID NO: 124 - protein, 6 aa, Artificial Sequence
YGYHWN

SEQ ID NO: 125 - protein, 6 aa, Artificial Sequence
RDYHWN

SEQ ID NO: 126 - protein, 6 aa, Artificial Sequence
RWYHWN

SEQ ID NO: 127 - protein, 6 aa, Artificial Sequence
NFYHWN

SEQ ID NO: 128 - protein, 6 aa, Artificial Sequence
RYYHWN

SEQ ID NO: 129 - protein, 14 aa, Artificial Sequence
WIRQFPGNKLEWIG

SEQ ID NO: 130 - protein, 14 aa, Artificial Sequence
WVRQFPGNKLEWIG

SEQ ID NO: 131 - protein, 14 aa, Artificial Sequence
WIQQFPGNKLEWIG

SEQ ID NO: 132 - protein, 14 aa, Artificial Sequence
WIRQLPGNKLEWIG

SEQ ID NO: 133 - protein, 14 aa, Artificial Sequence
WIRQFPGKKLEWIG

SEQ ID NO: 134 - protein, 14 aa, Artificial Sequence
WIRQFPGKGLEWIG

SEQ ID NO: 135 - protein, 14 aa, Artificial Sequence
WIRQFPGNKLVWMG

SEQ ID NO: 136 - protein, 14 aa, Artificial Sequence
WIRQFPGKSLEWIG

SEQ ID NO: 137 - protein, 14 aa, Artificial Sequence
WIRQFPGKRLEWMG

SEQ ID NO: 138 - protein, 14 aa, Artificial Sequence
WIRQFPGNELEWIG

SEQ ID NO: 139 - protein, 14 aa, Artificial Sequence
WIRQFPGNRLEWIG

SEQ ID NO: 140 - protein, 14 aa, Artificial Sequence
WIRQFPGNRLEWMG

SEQ ID NO: 141 - protein, 14 aa, Artificial Sequence
WIRQFPGNKLEWMG

SEQ ID NO: 142 - protein, 16 aa, Artificial Sequence
YISYDGSDHYNPSLEN

SEQ ID NO: 143 - protein, 16 aa, Artificial Sequence
YISYDGSVFYNPSLEN

SEQ ID NO: 144 - protein, 16 aa, Artificial Sequence
YISYDGSILYNPSLEN

SEQ ID NO: 145 - protein, 16 aa, Artificial Sequence
YISYDGTILYNPSLEN

SEQ ID NO: 146 - protein, 16 aa, Artificial Sequence
YISYDGTVLYNPSLEN

SEQ ID NO: 147 - protein, 16 aa, Artificial Sequence
YISYDGNVLYNPSLEN

SEQ ID NO: 148 - protein, 16 aa, Artificial Sequence
YISYDGTSLYNPSLEN

SEQ ID NO: 149 - protein, 16 aa, Artificial Sequence
YISYDGSVLYNPSLEN

SEQ ID NO: 150 - protein, 16 aa, Artificial Sequence
YISYDGNILYNPSLEN

SEQ ID NO: 151 - protein, 16 aa, Artificial Sequence
YISYDGTNLYNPSLEN

SEQ ID NO: 152 - protein, 16 aa, Artificial Sequence
YISYDGSNLYNPSLEN

SEQ ID NO: 153 - protein, 16 aa, Artificial Sequence
YISYDGTVHYNPSLEN

SEQ ID NO: 154 - protein, 16 aa, Artificial Sequence
YISYDGTIRYNPSLEN

SEQ ID NO: 155 - protein, 16 aa, Artificial Sequence
YISYDGSVLYNPSLKS

SEQ ID NO: 156 - protein, 16 aa, Artificial Sequence
YISYDGSVLYNPSLKG

SEQ ID NO: 157 - protein, 16 aa, Artificial Sequence
YIAYDGVQSYNPSLKG

SEQ ID NO: 158 - protein, 16 aa, Artificial Sequence
YIGYDGAVQYNPSLKS

SEQ ID NO: 159 - protein, 16 aa, Artificial Sequence
YISYNGSVLYNPSLKS

SEQ ID NO: 160 - protein, 16 aa, Artificial Sequence
YISYDGSRLYNPSLKS

SEQ ID NO: 161 - protein, 32 aa, Artificial Sequence
RITITRDTSKNQFSLILRSVTAEDTAIYYCAS

SEQ ID NO: 162 - protein, 32 aa, Artificial Sequence
RVTITRDTSKNQFFLKLSSVTAEDTAKYYCAS

SEQ ID NO: 163 - protein, 32 aa, Artificial Sequence
RVTITRDTSKNQFFLKLSSVTAEDTARYYCAS

SEQ ID NO: 164 - protein, 32 aa, Artificial Sequence
RITISRDTSKNQFFLKLRSVTAEDTAKYFCAS

SEQ ID NO: 165 - protein, 32 aa, Artificial Sequence
RVSITRDTSKNQFFLILRSVTAEDTAIYYCAS

SEQ ID NO: 166 - protein, 32 aa, Artificial Sequence
RVTITRDTSKNQFFLKLRSVTAEDTAIYYCAS

SEQ ID NO: 167 - protein, 32 aa, Artificial Sequence
RVSITRDTSKNQFFLKLSSVTAEDTAKYFCAS

SEQ ID NO: 168 - protein, 32 aa, Artificial Sequence
RVTITRDTSKNQFFLKLRSVTAEDTAIYFCAS

SEQ ID NO: 169 - protein, 32 aa, Artificial Sequence
RVTISVDTSKNQFSLKLSSVTAEDTAVYYCAS

SEQ ID NO: 170 - protein, 32 aa, Artificial Sequence
RVSISRDISKNQFFLKLSSVTAADTAVYFCAS

SEQ ID NO: 171 - protein, 32 aa, Artificial Sequence
RITITRDTSKNQFFLKLRSVTAEDTAVYYCAS

SEQ ID NO: 172 - protein, 32 aa, Artificial Sequence
RVSITRDTSKNQFFLKLRSVTAEDTAIYFCAS

SEQ ID NO: 173 - protein, 32 aa, Artificial Sequence
RITITRDTSKNQFFLKLRSVTAEDTAKYYCAS

SEQ ID NO: 174 - protein, 32 aa, Artificial Sequence
RVTITRDTSKNQFFLILRSVTAEDTAKYYCAS

SEQ ID NO: 175 - protein, 32 aa, Artificial Sequence
RVTITRDTSKNQFFLKLRSVTAEDTAKYYCAS

SEQ ID NO: 176 - protein, 32 aa, Artificial Sequence
RISITRDTSKNQFFLKLSSVTAEDTAKYFCAS

SEQ ID NO: 177 - protein, 32 aa, Artificial Sequence
RITITRDTSKNQFSLKLRSVTAEDTAVYYCAS

SEQ ID NO: 178 - protein, 32 aa, Artificial Sequence
RITITRDTSKNQFFLILRSVTAEDTAIYYCAS

SEQ ID NO: 179 - protein, 32 aa, Artificial Sequence
RVTISVDTSKNQFSLKLSSVTTEDTAVYYCAS

SEQ ID NO: 180 - protein, 4 aa, Artificial Sequence
GFDH

SEQ ID NO: 181 - protein, 4 aa, Artificial Sequence
GFDY

SEQ ID NO: 182 - protein, 4 aa, Artificial Sequence
GFDT

SEQ ID NO: 183 - protein, 11 aa, Artificial Sequence
WGQGTTLTVSS

SEQ ID NO: 184 - protein, 11 aa, Artificial Sequence
WGQGTLVTVSS

SEQ ID NO: 185 - protein, 11 aa, Artificial Sequence
WGQGTMLTVSS

SEQ ID NO: 186 - protein, 113 aa, Artificial Sequence
DVVMTQSPLSLPVTLGEPASISCRSNQSLVHSYGDTYLHWYLQKPGQSPKLLIYKVSNRFSGVPDRFSGSGSGTDFTLKISRVETEDVGVYYCSQNTHVPYTFGGGTKLEIKR

SEQ ID NO: 187 - protein, 113 aa, Artificial Sequence
DVVMTQSPLSLPVTLGEPASISCRSSQSLVHSYGDTYLHWYLQKPGQSPKLLIYKVSNRFSGVPDRFSGSGSGTDFTLKISRVETEDLGVYYCSQNTHVPYTFGGGTKLEIKR

SEQ ID NO: 188 - protein, 113 aa, Artificial Sequence
DVVMTQSPLSLPVTLGEPASISCRSSQSLVHSYGDTYLHWYLQKPGQSPKLLIYKVSNRFSGVPDRFSGSGSGTDFTLKISRVETEDVGVYYCSQNTHVPYTFGGGTKLEIKR

SEQ ID NO: 189 - protein, 113 aa, Artificial Sequence
DIVMTQSPLSLPVTLGEPASISCRSSQSLVHSYGDTYLHWYLQKPGQSPQLLIYKVSNRFSGVPDRFSGSGSGTDFTLKISRVETEDVGVYYCSQNTHVPYTFGGGTKLEIKR

SEQ ID NO: 190 - protein, 113 aa, Artificial Sequence
DVVMTQSPLSLPVTLGEPASISCRSSQSLVHSYGDTYLHWYLQKPGQSPQLLIYKVSNRFSGVPDRFSGSGSGTDFTLKISRVETEDLGVYYCSQNTHVPYTFGGGTKLEIKR

SEQ ID NO: 191 - protein, 113 aa, Artificial Sequence
DVVMTQSPLSLPVTLGEPASISCRSSQSLVHSYGDTYLHWYLQKPGQSPKLLIYKVSNRFSGVPDRFSGSGSGTDFTLKISRVETEDLGVYYCSQNTHLPYTFGGGTKLEIKR

SEQ ID NO: 192 - protein, 113 aa, Artificial Sequence
DVVMTQSPLSLPVTLGEPASISCRSSQSLVHSYGDTYLHWYLQKPGQSPQLLIYKVSNRFSGVPDRFSGSGSGTDFTLKISRVEAEDVGVYYCSQNTHVPYTFGQGTKLEIKR

SEQ ID NO: 193 - protein, 113 aa, Artificial Sequence
DVVMTQTPLSLPVNLGEPASISCRSSQSLVHSYGDTYLHWYLQKPGQSPKLLIYKVSNRFSGVPDRFSGSGSGTDFTLKISRVEAEDLGVYFCSQNTHVPYTFGGGTKLEIKR

SEQ ID NO: 194 - protein, 113 aa, Artificial Sequence
DVVMTQSPLSLPVTLGEPASISCRSSQSLVHSYGDTYLHWYLQKPGQSPQLLIYKVSNRFSGVPDRFSGSGSGTDFTLKISRVEAEDVGVYYCGQNAKTPYTFGQGTKLEIKR

SEQ ID NO: 195 - protein, 113 aa, Artificial Sequence
DVVMTQSPLSLPVTLGEPASISCRSSQSLVHSYGDTYLHWYLQKPGQSPQLLIYKVSNRFSGVPDRFSGSGSGTDFTLKISRVEAEDVGVYYCGQNARVPYTFGQGTKLEIKR

SEQ ID NO: 196 - protein, 113 aa, Artificial Sequence
DVVMTQSPLSLPVTLGEPASISCRSSQSLVHSYGDTYLHWYLQKPGQSPQLLIYKVSNRFSGVPDRFSGSGSGTDFTLKISRVEAEDVGVYYCSQNSYVPYTFGQGTKLEIKR

SEQ ID NO: 197 - protein, 113 aa, Artificial Sequence
DVVMTQSPLSLPVTLGEPASISCRSSQSLVHSYGDTYLHWYLQKPGQSPQLLIYKVSNRFSGVPDRFSGSGSGTDFTLKISRVEAEDVGVYYCSQNTIPPYTFGQGTKLEIKR

SEQ ID NO: 198 - protein, 113 aa, Artificial Sequence
DVVMTQSPLSLPVTLGEPASISCRSSQSLVHSYGDTYLHWYLQKPGQSPQLLIYKVSNRFSGVPDRFSGSGSGTDFTLKISRVEAEDVGVYYCGQNSMAPYTFGQGTKLEIKR

SEQ ID NO: 199 - protein, 113 aa, Artificial Sequence
DVVMTQSPLSLPVTLGEPASISCRSSQSLVHPYGPTYLHWYLQKPGQSPQLLIYKVSKRNSGVPDRFSGSGSGTDFTLKISRVEAEDVGVYYCSQNTHVPYTFGQGTKLEIKR

SEQ ID NO: 200 - protein, 113 aa, Artificial Sequence
DVVMTQSPLSLPVTLGEPASISCRSSQSLVHPYGPTYLHWYLQKPGQSPQLLIYKVSNRFSGVPDRFSGSGSGTDFTLKISRVEAEDVGVYYCSQNTHVPYTFGQGTKLEIKR

SEQ ID NO: 201 - protein, 113 aa, Artificial Sequence
DVVMTQSPLSLPVTLGEPASISCRSSQSLVHTYGNTYLHWYLQKPGQSPQLLIYKVSNRFSGVPDRFSGSGSGTDFTLKISRVEAEDVGVYYCSQNTHVPYTFGQGTKLEIKR

SEQ ID NO: 202 - protein, 113 aa, Artificial Sequence
DVVMTQSPLSLPVTLGEPASISCRSSQSLVHPYGSTYLHWYLQKPGQSPQLLIYKVSNRFSGVPDRFSGSGSGTDFTLKISRVEAEDVGVYYCSQNTHVPYTFGQGTKLEIKR

SEQ ID NO: 203 - protein, 113 aa, Artificial Sequence
DVVMTQSPLSLPVTLGEPASISCRSSQSLVHRYGTTYLHWYLQKPGQSPQLLIYKVSNRFSGVPDRFSGSGSGTDFTLKISRVEAEDVGVYYCSQNTHVPYTFGQGTKLEIKR

SEQ ID NO: 204 - protein, 113 aa, Artificial Sequence
DVVMTQSPLSLPVTLGEPASISCRSSQSLVHPYGATYLHWYLQKPGQSPQLLIYKASQRNSGVPDRFSGSGSGTDFTLKISRVEAEDVGVYYCSQNTHVPYTFGQGTKLEIKR

SEQ ID NO: 205 - protein, 113 aa, Artificial Sequence
DVVMTQSPLSLPVTLGEPASISCRSSQSLVHSYGDTYLHWYLQKPGQSPKLLIYKVSNRFSGVPDRFSGSGSGTDFTLKISRVEAEDVGVYYCSQNTHVPYTFGQGTKLEIKR

SEQ ID NO: 206 - protein, 113 aa, Artificial Sequence
DVVMTQSPLSLPVTLGEPASISCRSSQSLVHPYGPTYLHWYLQKPGQSPQLLIYKVSNRFSGVPDRFSGSGSGTDFTLKISRVEAEDVGVYYCGQNAHLPYTFGQGTKLEIKR

SEQ ID NO: 207 - protein, 113 aa, Artificial Sequence
DIVMTQSPLSLPVTLGEPASISCRSSQSLVHSYGDTYLHWYLQKPGQSPQLLIYKVSNRFSGVPDRFSGSGSGTDFTLKISRVETEDLGVYFCSQNTHVPYTFGGGTKLEIKR

SEQ ID NO: 208 - protein, 113 aa, Artificial Sequence
DIVMTQSPLSLPVTLGEQASISCRSSQSLVHSYGDTYLHWYLQKPGQSPQLLIYKVSNRFSGVPDRFSGSGSGTDFTLKISRVETEDLGVYFCSQNTHVPYTFGGGTKLEIKR

SEQ ID NO: 209 - protein, 113 aa, Artificial Sequence
DVVMTQSPLSLPVTLGEPASISCRSSQSLVHPYGRTYLHWYLQKPGQSPQLLIYRSSHRNSGVPDRFSGSGSGTDFTLKISRVEAEDVGVYYCSQNTHVPYTFGQGTKLEIKR

SEQ ID NO: 210 - protein, 113 aa, Artificial Sequence
DIVMTQSPLSLPVTLGEQASISCRSSQSLVHSYGDTYLHWYLQKPGQSPKLLIYKVSNRFSGVPDRFSGSGSGTDFTLKISRVETEDLGVYFCSQNTHVPYTFGGGTKLEIKR

SEQ ID NO: 211 - protein, 113 aa, Artificial Sequence
DIVMTQSPLSLPVTLGEQASISCRSSQSLVHSYGDTYLHWYLQKPGQSPKLLIYKVSNRFSGVPDRFSGSGSGTDFTLKISRVDTEDLGVYFCSQNTHVPYTFGGGTKLEIKR

SEQ ID NO: 212 - protein, 113 aa, Artificial Sequence
DIVMTQSPLSLPVTLGEQASISCRSSQSLVHSYGDTYLHWYLQKPGQSPKLLIYKVSNRFSGVPDRFSGSGSGTDFTLKISRVETEDLGVYYCSQNTHVPYTFGGGTKLEIKR

SEQ ID NO: 213 - protein, 113 aa, Artificial Sequence
DVVMTQSPLSLPVTLGEQASISCRSSQSLVHSYGDTYLHWYLQKPGQSPKLLIYKVSNRFSGVPDRFSGSGSGTDFTLKISRVETEDLGVYYCSQNTHVPYTFGGGTKLEIKR

SEQ ID NO: 214 - protein, 113 aa, Artificial Sequence
DIVMTQSPLSLPVTPGEPASISCRSSQSLVHSYGDTYLHWYLQKPGQSPKLLIYKVSNRFSGVPDRFSGSGSGTDFTLKISRVETEDVGVYFCSQNTHVPYTFGGGTKLEIKR

SEQ ID NO: 215 - protein, 23 aa, Artificial Sequence
DVVMTQSPLSLPVTLGEPASISC

SEQ ID NO: 216 - protein, 23 aa, Artificial Sequence
DIVMTQSPLSLPVTLGEPASISC

SEQ ID NO: 217 - protein, 23 aa, Artificial Sequence
DVVMTQTPLSLPVNLGEPASISC

SEQ ID NO: 218 - protein, 23 aa, Artificial Sequence
DIVMTQSPLSLPVTLGEQASISC

SEQ ID NO: 219 - protein, 23 aa, Artificial Sequence
DVVMTQSPLSLPVTLGEQASISC

SEQ ID NO: 220 - protein, 23 aa, Artificial Sequence
DIVMTQSPLSLPVTPGEPASISC

SEQ ID NO: 221 - protein, 15 aa, Artificial Sequence
WYLQKPGQSPKLLIY

SEQ ID NO: 222 - protein, 15 aa, Artificial Sequence
WYLQKPGQSPQLLIY

SEQ ID NO: 223 - protein, 32 aa, Artificial Sequence
GVPDRFSGSGSGTDFTLKISRVETEDVGVYYC

SEQ ID NO: 224 - protein, 32 aa, Artificial Sequence
GVPDRFSGSGSGTDFTLKISRVETEDLGVYYC

SEQ ID NO: 225 - protein, 32 aa, Artificial Sequence
GVPDRFSGSGSGTDFTLKISRVEAEDVGVYYC

SEQ ID NO: 226 - protein, 32 aa, Artificial Sequence
GVPDRFSGSGSGTDFTLKISRVEAEDLGVYFC

SEQ ID NO: 227 - protein, 32 aa, Artificial Sequence
GVPDRFSGSGSGTDFTLKISRVETEDLGVYFC

SEQ ID NO: 228 - protein, 32 aa, Artificial Sequence
GVPDRFSGSGSGTDFTLKISRVDTEDLGVYFC

SEQ ID NO: 229 - protein, 32 aa, Artificial Sequence
GVPDRFSGSGSGTDFTLKISRVETEDVGVYFC

SEQ ID NO: 230 - protein, 11 aa, Artificial Sequence
FGGGTKLEIKR

SEQ ID NO: 231 - protein, 11 aa, Artificial Sequence
FGQGTKLEIKR

SEQ ID NO: 232 - protein, 16 aa, Artificial Sequence
RSNQSLVHSYGDTYLH

SEQ ID NO: 233 - protein, 16 aa, Artificial Sequence
RSSQSLVHSYGDTYLH

SEQ ID NO: 234 - protein, 16 aa, Artificial Sequence
RSSQSLVHPYGPTYLH

SEQ ID NO: 235 - protein, 16 aa, Artificial Sequence
RSSQSLVHTYGNTYLH

SEQ ID NO: 236 - protein, 16 aa, Artificial Sequence
RSSQSLVHPYGSTYLH

SEQ ID NO: 237 - protein, 16 aa, Artificial Sequence
RSSQSLVHRYGTTYLH

SEQ ID NO: 238 - protein, 16 aa, Artificial Sequence
RSSQSLVHPYGATYLH

SEQ ID NO: 239 - protein, 16 aa, Artificial Sequence
RSSQSLVHPYGRTYLH

SEQ ID NO: 240 - protein, 7 aa, Artificial Sequence
KVSNRFS

SEQ ID NO: 241 - protein, 7 aa, Artificial Sequence
KVSKRNS

SEQ ID NO: 242 - protein, 7 aa, Artificial Sequence
KASQRNS

SEQ ID NO: 243 - protein, 7 aa, Artificial Sequence
RSSHRNS

SEQ ID NO: 244 - protein, 9 aa, Artificial Sequence
SQNTHVPYT

SEQ ID NO: 245 - protein, 9 aa, Artificial Sequence
SQNTHLPYT

SEQ ID NO: 246 - protein, 9 aa, Artificial Sequence
GQNAKTPYT

SEQ ID NO: 247 - protein, 9 aa, Artificial Sequence
GQNARVPYT

SEQ ID NO: 248 - protein, 9 aa, Artificial Sequence
SQNSYVPYT

SEQ ID NO: 249 - protein, 9 aa, Artificial Sequence
SQNTIPPYT

SEQ ID NO: 250 - protein, 9 aa, Artificial Sequence
GQNSMAPYT

SEQ ID NO: 251 - protein, 9 aa, Artificial Sequence
GQNAHLPYT

SEQ ID NO: 252 - DNA, 59 bp, Artificial Sequence
  misc_feature (38)..(39): n is a, c, g, or t
gactgtgagagttgtgccttggccccagtggtcaaavnnactcgcacagtaatatatgg

SEQ ID NO: 253 - DNA, 43 bp, Artificial Sequence
gcacaactctcacagtctcctcaggaggtggcggatctggagg

SEQ ID NO: 254 - DNA, 51 bp, Artificial Sequence
gttattactcgtggcccagccggccatggcagaggtgcagctgcaggagtc

SEQ ID NO: 255 - DNA, 51 bp, Artificial Sequence
gtcgaccaggcccccgaggccccgttttatttccagcttggtcccccctcc

SEQ ID NO: 256 - DNA, 59 bp, Artificial Sequence
acggatctctagcgaattcatgggaaggcttacttcttcattcctgctactgattgtcc

SEQ ID NO: 257 - DNA, 38 bp, Artificial Sequence
tgggcccttgaagcttgctgaggagactgtgagagttg

SEQ ID NO: 258 - DNA, 43 bp, Artificial Sequence
ttttccttttgcggccgcttatttacccggagacagggagagg

SEQ ID NO: 259 - DNA, 59 bp, Artificial Sequence
cggatctctagcgaattcatgtctgtgccaactcaggtcctggggttgctgctgctgtg

SEQ ID NO: 260 - DNA, 40 bp, Artificial Sequence
acagatggtgcagccacagtccgttttatttccagcttgg

SEQ ID NO: 261 - DNA, 33 bp, Artificial Sequence
actgtggctgcaccatctgtcttcatcttcccg

SEQ ID NO: 262 - DNA, 52 bp, Artificial Sequence
aaacgggccctctagattaacactctcccctgttgaagctctttgtgacggg

SEQ ID NO: 263 - protein, 113 aa, Artificial Sequence
QVQLQESGPGLVKPSQTLSLTCAVSGSSITRGYHWNWIRQFPGKGLEWIGYISYDGSVLYNPSLKSRVTISVDTSKNQFSLKLSSVTTEDTAVYYCASGFDHWGQGTLVTVSS

SEQ ID NO: 264 - protein, 113 aa, Artificial Sequence
QVQLQESGPGLVKPSQTLSLTCAVSGYSISRGYHWNWIRQFPGNKLEWIGYISYDGSVLYNPSLENRVTITRDTSKNQFSLKLSSVTTEDTAVYYCASGFDHWGQGTLVTVSS

SEQ ID NO: 265 - protein, 113 aa, Artificial Sequence
QVQLQESGPGLVKPSQTLSLTCAVSGYSISYGYHWNWIRQFPGNKLEWIGYISYDGSVLYNPSLENRVTITRDTSKNQFSLKLSSVTAEDTAVYYCASGFDHWGQGTLVTVSS

SEQ ID NO: 266 - protein, 113 aa, Artificial Sequence
QVQLQESGPGLVKPSQTLSLTCAVSGSSITYGYHWNWIRQFPGNKLEWIGYISYDGSVLYNPSLENRVTITRDTSKNQFSLKLSSVTAEDTAVYYCASGFDHWGQGTLVTVSS

SEQ ID NO: 267 - protein, 113 aa, Artificial Sequence
QVQLQESGPGLVKPSQTLSLTCAVSGYSISSGYHWNWIRQFPGKGLEWIGYISYDGSVLYNPSLKSRVTISVDRSKNQFSLKLSSVTAEDTAVYYCASGFDHWGQGTLVTVSS

SEQ ID NO: 268 - protein, 113 aa, Artificial Sequence
QVQLQESGPGLVKPSQTLSLTCAVSGYSISRGYHWNWIRQFPGKGLEWIGYISYDGSVLYNPSLKSRVTVSVDTSKNQFSLKLSSVTTEDTAVYYCASGFDHWGQGTLVTVSS

SEQ ID NO: 269 - protein, 113 aa, Artificial Sequence
QVQLQESGPGLVKPSQTLSLTCAVSGYSISRGYHWNWIRQFPGKGLEWIGYISYDGSVLYNPSLKSRVTISVDTSKNQFSLKLSSVTTEDSAVYYCSSGFDHWGQGTLVTVSS

SEQ ID NO: 270 - protein, 113 aa, Artificial Sequence
QVQLQESGPGLVKPSQTLSLTCAVSGYSISRGYHWNWIRQFPGKGLEWIGYISYDGSVLYNPSLKSRVTISVDTSKNQFSLKLSSVTTEDTAVYYCASGFDHWGHGTLVTVSS

SEQ ID NO: 271 - protein, 113 aa, Artificial Sequence
QVQLQESGPGLVKPSQTLSLTCAVSGYSISRGYHWNWIRQYPGKGLEWIGYISYDGSVLYNPSLKSRVAISVDTSKNQFSLKLSSVTAEDTAVYYCASGFDHWGQGTLVTVSS

SEQ ID NO: 272 - protein, 113 aa, Artificial Sequence
QVQLQESGPGLVKPSQTLSLSCAVSGYSISRGYHWNWIRQFPGKGLEWIGYISYDGSVLYNPSLKGRVTISVDTSKNQFSLKLSSVTAEDTAVYYCASGFDHWGQGTLVTVSS

SEQ ID NO: 273 - protein, 113 aa, Artificial Sequence
QVQLQESGPGLVKPSQTLSLTCAVSGYSISRGYHWNWIRQFPGKGLEWLGYISYDGSVLYNPSLKSRVTISVDTSKNQFSLKLSSVTAEDTAVYYCASGFDHWGQGTLVTVSS

SEQ ID NO: 274 - protein, 113 aa, Artificial Sequence
QVQLQESGPGLVKPSQTLSLTCAVSGYSISRGYHWNWIRQFPGKGLEWIGYISYDGSVLYNPSLKSRVTISEDTSKNQFSLKLSSVTAEDTAVYYCASGFDHWGQGTLVTVSS

SEQ ID NO: 275 - protein, 113 aa, Artificial Sequence
QVQLQESGPGLVKPSQTLSLTCAVSGYSISSGYHWNWIRQFPGKGLEWIGYISYDGSVLYNPSLKSRVTISMDTSKNHFSLKLSSVTAEDTAVYYCASGFDHWGQGTLVTVSS

SEQ ID NO: 276 - protein, 113 aa, Artificial Sequence
QVQLQESGPGRVKPSQTLSLTCAVSGYSISRGYHWNWIRQFPGKGLEWIGYISYDGSVLYNPSLKSRVTISVDTSKNQFSLKLSSVTTEDTAVYYCASGFDHWGQGTLVTVSS

SEQ ID NO: 277 - protein, 113 aa, Artificial Sequence
QVQLQESGPGLVKPSQTLSLTCAVSGYSISRGYHWNWIRQFPGKGLEWIGYISYDGSVLFNPSLKSRVTISVDRSKNQFSLKLSSVTAEDTAVYYCASGFDHWGPGTQVTVSS

SEQ ID NO: 278 - protein, 113 aa, Artificial Sequence
QVQLQESGPGLVKPSQTLSLSCAVSGYSISSGYHWNWIRQFPGKGLEWIGYISYDGSVLYNPSLKSRVTIGVDTSKNQFSLKLSSVTAEDTAVYYCASGFDHWGQGTLVTVSS

SEQ ID NO: 279 - protein, 113 aa, Artificial Sequence
QVQLQESGPGLVKPSQTLSLTCAVSGYSISRGYHWNWIRQFPGKGLEWIGYISYDGSVLYNPSLKSRVTISVDTSKNQFSLKLRSVTDEDSAVYYCASGFDHWGQGTLVTVSS

SEQ ID NO: 280 - protein, 30 aa, Artificial Sequence
QVQLQESGPGLVKPSQTLSLTCAVSGSSIT

SEQ ID NO: 281 - protein, 30 aa, Artificial Sequence
QVQLQESGPGLVKPSQTLSLSCAVSGYSIS

SEQ ID NO: 282 - protein, 30 aa, Artificial Sequence
QVQLQESGPGRVKPSQTLSLTCAVSGYSIS

SEQ ID NO: 283 - protein, 14 aa, Artificial Sequence
WIRQYPGKGLEWIG

SEQ ID NO: 284 - protein, 14 aa, Artificial Sequence
WIRQFPGKGLEWLG

SEQ ID NO: 285 - protein, 16 aa, Artificial Sequence
YISYDGSVLFNPSLKS

SEQ ID NO: 286 - protein, 32 aa, Artificial Sequence
RVTITRDTSKNQFSLKLSSVTTEDTAVYYCAS

SEQ ID NO: 287 - protein, 32 aa, Artificial Sequence
RVTITRDTSKNQFSLKLSSVTAEDTAVYYCAS

SEQ ID NO: 288 - protein, 32 aa, Artificial Sequence
RVTISVDRSKNQFSLKLSSVTAEDTAVYYCAS

SEQ ID NO: 289 - protein, 32 aa, Artificial Sequence
RVTVSVDTSKNQFSLKLSSVTTEDTAVYYCAS

SEQ ID NO: 290 - protein, 32 aa, Artificial Sequence
RVTISVDTSKNQFSLKLSSVTTEDSAVYYCSS

SEQ ID NO: 291 - protein, 32 aa, Artificial Sequence
RVAISVDTSKNQFSLKLSSVTAEDTAVYYCAS

SEQ ID NO: 292 - protein, 32 aa, Artificial Sequence
RVTISEDTSKNQFSLKLSSVTAEDTAVYYCAS

SEQ ID NO: 293 - protein, 32 aa, Artificial Sequence
RVTISMDTSKNHFSLKLSSVTAEDTAVYYCAS

SEQ ID NO: 294 - protein, 32 aa, Artificial Sequence
RVTIGVDTSKNQFSLKLSSVTAEDTAVYYCAS

SEQ ID NO: 295 - protein, 32 aa, Artificial Sequence
RVTISVDTSKNQFSLKLRSVTDEDSAVYYCAS

SEQ ID NO: 296 - protein, 11 aa, Artificial Sequence
WGHGTLVTVSS

SEQ ID NO: 297 - protein, 11 aa, Artificial Sequence
WGPGTQVTVSS

SEQ ID NO: 298 - protein, 113 aa, Artificial Sequence
DVVMTQSPISLPVTLGEPASISCRSSQSLVHPYGSTYLHWYLQKPGQSPQLLIYKVSNRFSGVPDRFSGSGSGTDFTLKISRVEAEDVGVYYCSQNTHVPYTFGQGTKLEIKR

SEQ ID NO: 299 - protein, 113 aa, Artificial Sequence
DVVMTQSPLSLPVTLGEPASISCRSSQSLVHPYGSTYLHWYLQKPGQPPQLLIYKVSNRFSGVPDRFSGSGSGTDFTLKISRVEAEDVGVYYCSQNTHVPYTFGQGTKLEIKR

SEQ ID NO: 300 - protein, 113 aa, Artificial Sequence
DVVMTQSPLSLSVTLGEPASISCRSSQSLVHPYGPTYLHWYLQKPGQSPQLLIYKVSNRFSGVPDRFSGSGSGTDYTLKISRVEAEDVGVYYCSQNTHVPYTFGQGTKLEIKR

SEQ ID NO: 301 - protein, 113 aa, Artificial Sequence
DVVMTQSPLSLPVTLGEPASISCRSSQSLVHSYGDTYLHWYLQKPGQSPKLLIYKVSNRFSGVPDRFSGSGSGTDYTLKISRVEAEDVGVYYCSQNTHVPYTFGQGTKLEIKR

SEQ ID NO: 302 - protein, 113 aa, Artificial Sequence
DVVMTQSPLSLPVTLGEPASISCRSSQSLVHPYGPTYLHWYLQKPGQSPQLLIYKVSNRFSGVPDRFSGSGSGTEFTLKISRVEAEDVGAYYCSQNTHVPYTFGQGTKLEIKR

SEQ ID NO: 303 - protein, 113 aa, Artificial Sequence
DVVMTQSPLSLPVTLGEPASISCRSSQSLVHPFGPTYLHWYLQKPGQSPKLLIYKVSNRFSGVPDRFSGSGSGTDFTLKISRVEAEDVGVYYCSQNTHVPYTFGQGTKLEIKR

SEQ ID NO: 304 - protein, 113 aa, Artificial Sequence
DVVMTQSPLSLPVTLGEPASISCRSSQSLAHPYGSTYLHWYLQKPGQSPQLLIYKVSNRFSGVPDRFSGSGSGTDFTLKISRVEAEDVGVYYCSQNTHVPYTFGQGTKLEIKR

SEQ ID NO: 305 - protein, 113 aa, Artificial Sequence
DVVMTQSPLSLPVTLGEPASISCRSSQSLVHSYGDTYLHWYLQKPGQSPQLLIYKVSNRFSGVPDRFSGSGSGTDFTLKISRVEAEDVGVYYCSQNTHVPYTFGQGTRLEIKR

SEQ ID NO: 306 - protein, 113 aa, Artificial Sequence
DVVMTQSPLSLPVTLGEPASISCRSSQSLVHPYGPTYLHWYLQKPGQSPQLLIYKVSNRFSGVPDRFSGGGSGTDFTLKISRVEAEDVGVYYCSQNTHVPYTFGQGTKLEIKR

SEQ ID NO: 307 - protein, 113 aa, Artificial Sequence
DVVMTQSPLSLPVTLGEPASISCRSSQSLVHPYGPTYLHWYLQKPGQSPQLLVYKVSNRFSGVPDRFSGSGSGTDFTLKISRVEAEDVGVYYCSQNTHVPYTFGQGTKLEIKR

SEQ ID NO: 308 - protein, 113 aa, Artificial Sequence
DVVMTQSPLSLPVTLGEPASISCRSSQSLVHPYGSTYFHWYLQKPGQSPQLLIYKVSNRFSGVPDRFSGSGSGTDFTLKISRVEAEDGGVYYCSQNTHVPYTFGQGTKLEIKR

SEQ ID NO: 309 - protein, 23 aa, Artificial Sequence
DVVMTQSPISLPVTLGEPASISC

SEQ ID NO: 310 - protein, 23 aa, Artificial Sequence
DVVMTQSPLSLSVTLGEPASISC

SEQ ID NO: 311 - protein, 15 aa, Artificial Sequence
WYLQKPGQPPQLLIY

SEQ ID NO: 312 - protein, 15 aa, Artificial Sequence
WYLQKPGQSPQLLVY

SEQ ID NO: 313 - protein, 32 aa, Artificial Sequence
GVPDRFSGSGSGTDYTLKISRVEAEDVGVYYC

SEQ ID NO: 314 - protein, 32 aa, Artificial Sequence
GVPDRFSGSGSGTEFTLKISRVEAEDVGAYYC

SEQ ID NO: 315 - protein, 32 aa, Artificial Sequence
GVPDRFSGGGSGTDFTLKISRVEAEDVGVYYC

SEQ ID NO: 316 - protein, 32 aa, Artificial Sequence
GVPDRFSGSGSGTDFTLKISRVEAEDGGVYYC

SEQ ID NO: 317 - protein, 11 aa, Artificial Sequence
FGQGTRLEIKR

SEQ ID NO: 318 - protein, 16 aa, Artificial Sequence
RSSQSLVHPFGPTYLH

SEQ ID NO: 319 - protein, 16 aa, Artificial Sequence
RSSQSLAHPYGSTYLH

SEQ ID NO: 320 - protein, 16 aa, Artificial Sequence
RSSQSLVHPYGSTYFH